European Patent Application EP 4 573 926 A1, published June 25, 2025. Title: Composition for preventing, ameliorating or treating parkinson's disease comprising osmotin protein as effective component. Applicant: INDUSTRY-ACADEMIC COOPERATION FOUNDATION GYEONGSANG NATIONAL UNIVERSITY. Application KR. The sequence listing filed with the application follows.

SEQUENCE LISTING (1 sequence)

SEQ ID NO: 1 - protein, 243 aa, Nicotiana tabacum
MGNLRSSFVFFLLALVTYTYAATIEVRNNCPYTVWAASTPIGGGRRLDRGQTWVINAPRGTKMARVWGRTNCNFNAAGRGTCQTGDCGGVLQCTGWGKPPNTLAEYALDQFSGLDFWDISLLDGFNIPITFPTNPSGGKCHALCTAINGECPAELRVPGGCNNPCTTFGGQQYCCTQRPCGPTFFSKFFKQRCPDAYSYPQDDPTSTFTCPGGSTNYRVIFCPNGQAHPNFPLEMPGSDEVAK